European Patent Specification EP 4 045 150 B1, published November 26, 2025. Title: IMMUNOGENIC COMPOUNDS FOR TREATMENT OF ADRENAL CANCER. Applicant: ENTEROME SA. The sequence listing filed with the application follows.

SEQUENCE LISTING (344 sequences)

SEQ ID NO: 1 - protein, 9 aa, Artificial Sequence
  peptide
ALGCLYTFV

SEQ ID NO: 2 - protein, 9 aa, Artificial Sequence
  peptide
AMGCLYTFI

SEQ ID NO: 3 - protein, 9 aa, Artificial Sequence
  peptide
AMGCLYTFV

SEQ ID NO: 4 - protein, 9 aa, Artificial Sequence
  peptide
CMYTFLISV

SEQ ID NO: 5 - protein, 9 aa, Artificial Sequence
  peptide
CSDDGIWSI

SEQ ID NO: 6 - protein, 9 aa, Artificial Sequence
  peptide
CSDDGIWSL

SEQ ID NO: 7 - protein, 9 aa, Artificial Sequence
  peptide
CSDDGIWSV

SEQ ID NO: 8 - protein, 9 aa, Artificial Sequence
  peptide
FASDYKDFY

SEQ ID NO: 9 - protein, 9 aa, Artificial Sequence
  peptide
FIGCLYTFI

SEQ ID NO: 10 - protein, 9 aa, Artificial Sequence
  peptide
FIGCLYTFL

SEQ ID NO: 11 - protein, 9 aa, Artificial Sequence
  peptide
FIGCLYTFV

SEQ ID NO: 12 - protein, 9 aa, Artificial Sequence
  peptide
FIVKPLPPV

SEQ ID NO: 13 - protein, 9 aa, Artificial Sequence
  peptide
FLCSWKPGI

SEQ ID NO: 14 - protein, 9 aa, Artificial Sequence
  peptide
FLCSWKPGL

SEQ ID NO: 15 - protein, 9 aa, Artificial Sequence
  peptide
FLCSWKPGV

SEQ ID NO: 16 - protein, 9 aa, Artificial Sequence
  peptide
FLDDGIWSI

SEQ ID NO: 17 - protein, 9 aa, Artificial Sequence
  peptide
FLDDGIWSL

SEQ ID NO: 18 - protein, 9 aa, Artificial Sequence
  peptide
FLDDGIWSV

SEQ ID NO: 19 - protein, 9 aa, Artificial Sequence
  peptide
FLDHALQCV

SEQ ID NO: 20 - protein, 9 aa, Artificial Sequence
  peptide
FLDKQCWEV

SEQ ID NO: 21 - protein, 9 aa, Artificial Sequence
  peptide
FLFYWYEGI

SEQ ID NO: 22 - protein, 9 aa, Artificial Sequence
  peptide
FLFYWYEGL

SEQ ID NO: 23 - protein, 9 aa, Artificial Sequence
  peptide
FLFYWYEGV

SEQ ID NO: 24 - protein, 9 aa, Artificial Sequence
  peptide
FLGCLYTFI

SEQ ID NO: 25 - protein, 9 aa, Artificial Sequence
  peptide
FLGCLYTFL

SEQ ID NO: 26 - protein, 9 aa, Artificial Sequence
  peptide
FLGCLYTFV

SEQ ID NO: 27 - protein, 9 aa, Artificial Sequence
  peptide
FLISTTFGI

SEQ ID NO: 28 - protein, 9 aa, Artificial Sequence
  peptide
FLISTTFGL

SEQ ID NO: 29 - protein, 9 aa, Artificial Sequence
  peptide
FLISTTFGV

SEQ ID NO: 30 - protein, 9 aa, Artificial Sequence
  peptide
FLNETYTLK

SEQ ID NO: 31 - protein, 9 aa, Artificial Sequence
  peptide
FLPFGFILV

SEQ ID NO: 32 - protein, 9 aa, Artificial Sequence
  peptide
FLSDYKDFY

SEQ ID NO: 33 - protein, 9 aa, Artificial Sequence
  peptide
FLTNYNLFY

SEQ ID NO: 34 - protein, 9 aa, Artificial Sequence
  peptide
FLVKPLPPI

SEQ ID NO: 35 - protein, 9 aa, Artificial Sequence
  peptide
FLVKPLPPL

SEQ ID NO: 36 - protein, 9 aa, Artificial Sequence
  peptide
FLVKPLPPV

SEQ ID NO: 37 - protein, 9 aa, Artificial Sequence
  peptide
FLWKTIITK

SEQ ID NO: 38 - protein, 9 aa, Artificial Sequence
  peptide
FLWQPPLSI

SEQ ID NO: 39 - protein, 9 aa, Artificial Sequence
  peptide
FLWQPPLSL

SEQ ID NO: 40 - protein, 9 aa, Artificial Sequence
  peptide
FLWQPPLSV

SEQ ID NO: 41 - protein, 9 aa, Artificial Sequence
  peptide
FLYLLCSWK

SEQ ID NO: 42 - protein, 9 aa, Artificial Sequence
  peptide
FLYTFLISI

SEQ ID NO: 43 - protein, 9 aa, Artificial Sequence
  peptide
FLYTFLISL

SEQ ID NO: 44 - protein, 9 aa, Artificial Sequence
  peptide
FLYTFLIST

SEQ ID NO: 45 - protein, 9 aa, Artificial Sequence
  peptide
FLYTFLISV

SEQ ID NO: 46 - protein, 9 aa, Artificial Sequence
  peptide
FMCSWKPGI

SEQ ID NO: 47 - protein, 9 aa, Artificial Sequence
  peptide
FMCSWKPGL

SEQ ID NO: 48 - protein, 9 aa, Artificial Sequence
  peptide
FMCSWKPGV

SEQ ID NO: 49 - protein, 9 aa, Artificial Sequence
  peptide
FMDDGIWSI

SEQ ID NO: 50 - protein, 9 aa, Artificial Sequence
  peptide
FMDDGIWSL

SEQ ID NO: 51 - protein, 9 aa, Artificial Sequence
  peptide
FMDDGIWSV

SEQ ID NO: 52 - protein, 9 aa, Artificial Sequence
  peptide
FMDHALQCV

SEQ ID NO: 53 - protein, 9 aa, Artificial Sequence
  peptide
FMDKQCWEV

SEQ ID NO: 54 - protein, 9 aa, Artificial Sequence
  peptide
FMFYWYEGI

SEQ ID NO: 55 - protein, 9 aa, Artificial Sequence
  peptide
FMFYWYEGL

SEQ ID NO: 56 - protein, 9 aa, Artificial Sequence
  peptide
FMFYWYEGV

SEQ ID NO: 57 - protein, 9 aa, Artificial Sequence
  peptide
FMGCLYTFI

SEQ ID NO: 58 - protein, 9 aa, Artificial Sequence
  peptide
FMGCLYTFL

SEQ ID NO: 59 - protein, 9 aa, Artificial Sequence
  peptide
FMGCLYTFV

SEQ ID NO: 60 - protein, 9 aa, Artificial Sequence
  peptide
FMISTTFGI

SEQ ID NO: 61 - protein, 9 aa, Artificial Sequence
  peptide
FMISTTFGL

SEQ ID NO: 62 - protein, 9 aa, Artificial Sequence
  peptide
FMISTTFGV

SEQ ID NO: 63 - protein, 9 aa, Artificial Sequence
  peptide
FMNETYTLK

SEQ ID NO: 64 - protein, 9 aa, Artificial Sequence
  peptide
FMPFGFILV

SEQ ID NO: 65 - protein, 9 aa, Artificial Sequence
  peptide
FMQDMCVYY

SEQ ID NO: 66 - protein, 9 aa, Artificial Sequence
  peptide
FMSDYKDFY

SEQ ID NO: 67 - protein, 9 aa, Artificial Sequence
  peptide
FMTGLLLRK

SEQ ID NO: 68 - protein, 9 aa, Artificial Sequence
  peptide
FMTNYNLFY

SEQ ID NO: 69 - protein, 9 aa, Artificial Sequence
  peptide
FMVIFVTGV

SEQ ID NO: 70 - protein, 9 aa, Artificial Sequence
  peptide
FMVKPLPPI

SEQ ID NO: 71 - protein, 9 aa, Artificial Sequence
  peptide
FMVKPLPPL

SEQ ID NO: 72 - protein, 9 aa, Artificial Sequence
  peptide
FMVKPLPPV

SEQ ID NO: 73 - protein, 9 aa, Artificial Sequence
  peptide
FMWKTIITK

SEQ ID NO: 74 - protein, 9 aa, Artificial Sequence
  peptide
FMWQPPLSI

SEQ ID NO: 75 - protein, 9 aa, Artificial Sequence
  peptide
FMWQPPLSL

SEQ ID NO: 76 - protein, 9 aa, Artificial Sequence
  peptide
FMWQPPLSV

SEQ ID NO: 77 - protein, 9 aa, Artificial Sequence
  peptide
FMYLLCSWK

SEQ ID NO: 78 - protein, 9 aa, Artificial Sequence
  peptide
FMYTFLISI

SEQ ID NO: 79 - protein, 9 aa, Artificial Sequence
  peptide
FMYTFLISL

SEQ ID NO: 80 - protein, 9 aa, Artificial Sequence
  peptide
FMYTFLIST

SEQ ID NO: 81 - protein, 9 aa, Artificial Sequence
  peptide
FMYTFLISV

SEQ ID NO: 82 - protein, 9 aa, Artificial Sequence
  peptide
FQWQPPLSV

SEQ ID NO: 83 - protein, 9 aa, Artificial Sequence
  peptide
FSDDGIWSI

SEQ ID NO: 84 - protein, 9 aa, Artificial Sequence
  peptide
FSDDGIWSL

SEQ ID NO: 85 - protein, 9 aa, Artificial Sequence
  peptide
FSDDGIWSV

SEQ ID NO: 86 - protein, 9 aa, Artificial Sequence
  peptide
FSDKQCWEI

SEQ ID NO: 87 - protein, 9 aa, Artificial Sequence
  peptide
FSDKQCWEL

SEQ ID NO: 88 - protein, 9 aa, Artificial Sequence
  peptide
FSDKQCWEV

SEQ ID NO: 89 - protein, 9 aa, Artificial Sequence
  peptide
FSDYKDFYI

SEQ ID NO: 90 - protein, 9 aa, Artificial Sequence
  peptide
FSDYKDFYL

SEQ ID NO: 91 - protein, 9 aa, Artificial Sequence
  peptide
FSDYKDFYV

SEQ ID NO: 92 - protein, 9 aa, Artificial Sequence
  peptide
FSSWAETTY

SEQ ID NO: 93 - protein, 9 aa, Artificial Sequence
  peptide
FTWKTIITK

SEQ ID NO: 94 - protein, 9 aa, Artificial Sequence
  peptide
FVQDMCVYY

SEQ ID NO: 95 - protein, 9 aa, Artificial Sequence
  peptide
LLTNYNLFY

SEQ ID NO: 96 - protein, 9 aa, Artificial Sequence
  peptide
LLWQPPLSV

SEQ ID NO: 97 - protein, 9 aa, Artificial Sequence
  peptide
LMTNYNLFY

SEQ ID NO: 98 - protein, 9 aa, Artificial Sequence
  peptide
LMWQPPLSI

SEQ ID NO: 99 - protein, 9 aa, Artificial Sequence
  peptide
LMWQPPLSL

SEQ ID NO: 100 - protein, 9 aa, Artificial Sequence
  peptide
LMWQPPLSV

SEQ ID NO: 101 - protein, 9 aa, Artificial Sequence
  peptide
RLIGSETWK

SEQ ID NO: 102 - protein, 9 aa, Artificial Sequence
  peptide
RMIGSETWK

SEQ ID NO: 103 - protein, 9 aa, Artificial Sequence
  peptide
VLNETYTLK

SEQ ID NO: 104 - protein, 9 aa, Artificial Sequence
  peptide
VMNETYTLK

SEQ ID NO: 105 - protein, 9 aa, Artificial Sequence
  peptide
WASDYKDFY

SEQ ID NO: 106 - protein, 9 aa, Artificial Sequence
  peptide
WLCSWKPGV

SEQ ID NO: 107 - protein, 9 aa, Artificial Sequence
  peptide
WLDDGIWSI

SEQ ID NO: 108 - protein, 9 aa, Artificial Sequence
  peptide
WLDDGIWSL

SEQ ID NO: 109 - protein, 9 aa, Artificial Sequence
  peptide
WLDDGIWSV

SEQ ID NO: 110 - protein, 9 aa, Artificial Sequence
  peptide
WLFYWYEGV

SEQ ID NO: 111 - protein, 9 aa, Artificial Sequence
  peptide
WLGCLYTFI

SEQ ID NO: 112 - protein, 9 aa, Artificial Sequence
  peptide
WLGCLYTFL

SEQ ID NO: 113 - protein, 9 aa, Artificial Sequence
  peptide
WLGCLYTFV

SEQ ID NO: 114 - protein, 9 aa, Artificial Sequence
  peptide
WLISTTFGL

SEQ ID NO: 115 - protein, 9 aa, Artificial Sequence
  peptide
WLISTTFGV

SEQ ID NO: 116 - protein, 9 aa, Artificial Sequence
  peptide
WLNETYTLK

SEQ ID NO: 117 - protein, 9 aa, Artificial Sequence
  peptide
WLSDYKDFY

SEQ ID NO: 118 - protein, 9 aa, Artificial Sequence
  peptide
WLTNYNLFY

SEQ ID NO: 119 - protein, 9 aa, Artificial Sequence
  peptide
WLVKPLPPV

SEQ ID NO: 120 - protein, 9 aa, Artificial Sequence
  peptide
WLWQPPLSI

SEQ ID NO: 121 - protein, 9 aa, Artificial Sequence
  peptide
WLWQPPLSL

SEQ ID NO: 122 - protein, 9 aa, Artificial Sequence
  peptide
WLWQPPLSV

SEQ ID NO: 123 - protein, 9 aa, Artificial Sequence
  peptide
WLYTFLISV

SEQ ID NO: 124 - protein, 9 aa, Artificial Sequence
  peptide
WMCSWKPGV

SEQ ID NO: 125 - protein, 9 aa, Artificial Sequence
  peptide
WMDDGIWSI

SEQ ID NO: 126 - protein, 9 aa, Artificial Sequence
  peptide
WMDDGIWSL

SEQ ID NO: 127 - protein, 9 aa, Artificial Sequence
  peptide
WMDDGIWSV

SEQ ID NO: 128 - protein, 9 aa, Artificial Sequence
  peptide
WMDKQCWEV

SEQ ID NO: 129 - protein, 9 aa, Artificial Sequence
  peptide
WMFYWYEGV

SEQ ID NO: 130 - protein, 9 aa, Artificial Sequence
  peptide
WMGCLYTFI

SEQ ID NO: 131 - protein, 9 aa, Artificial Sequence
  peptide
WMGCLYTFL

SEQ ID NO: 132 - protein, 9 aa, Artificial Sequence
  peptide
WMGCLYTFV

SEQ ID NO: 133 - protein, 9 aa, Artificial Sequence
  peptide
WMISTTFGI

SEQ ID NO: 134 - protein, 9 aa, Artificial Sequence
  peptide
WMISTTFGL

SEQ ID NO: 135 - protein, 9 aa, Artificial Sequence
  peptide
WMISTTFGV

SEQ ID NO: 136 - protein, 9 aa, Artificial Sequence
  peptide
WMNETYTLK

SEQ ID NO: 137 - protein, 9 aa, Artificial Sequence
  peptide
WMSDYKDFY

SEQ ID NO: 138 - protein, 9 aa, Artificial Sequence
  peptide
WMTNYNLFY

SEQ ID NO: 139 - protein, 9 aa, Artificial Sequence
  peptide
WMVKPLPPV

SEQ ID NO: 140 - protein, 9 aa, Artificial Sequence
  peptide
WMWKTIITK

SEQ ID NO: 141 - protein, 9 aa, Artificial Sequence
  peptide
WMWQPPLSI

SEQ ID NO: 142 - protein, 9 aa, Artificial Sequence
  peptide
WMWQPPLSL

SEQ ID NO: 143 - protein, 9 aa, Artificial Sequence
  peptide
WMWQPPLSV

SEQ ID NO: 144 - protein, 9 aa, Artificial Sequence
  peptide
WMYTFLISI

SEQ ID NO: 145 - protein, 9 aa, Artificial Sequence
  peptide
WMYTFLISL

SEQ ID NO: 146 - protein, 9 aa, Artificial Sequence
  peptide
WMYTFLISV

SEQ ID NO: 147 - protein, 9 aa, Artificial Sequence
  peptide
WSDDGIWSI

SEQ ID NO: 148 - protein, 9 aa, Artificial Sequence
  peptide
WSDDGIWSL

SEQ ID NO: 149 - protein, 9 aa, Artificial Sequence
  peptide
WSDDGIWSV

SEQ ID NO: 150 - protein, 9 aa, Artificial Sequence
  peptide
WSDKQCWEI

SEQ ID NO: 151 - protein, 9 aa, Artificial Sequence
  peptide
WSDKQCWEL

SEQ ID NO: 152 - protein, 9 aa, Artificial Sequence
  peptide
WSDKQCWEV

SEQ ID NO: 153 - protein, 9 aa, Artificial Sequence
  peptide
WSDYKDFYI

SEQ ID NO: 154 - protein, 9 aa, Artificial Sequence
  peptide
WSDYKDFYL

SEQ ID NO: 155 - protein, 9 aa, Artificial Sequence
  peptide
WSDYKDFYV

SEQ ID NO: 156 - protein, 9 aa, Artificial Sequence
  peptide
WVQDMCVYY

SEQ ID NO: 157 - protein, 9 aa, Artificial Sequence
  peptide
YASDYKDFY

SEQ ID NO: 158 - protein, 9 aa, Artificial Sequence
  peptide
YIGCLYTFI

SEQ ID NO: 159 - protein, 9 aa, Artificial Sequence
  peptide
YIGCLYTFL

SEQ ID NO: 160 - protein, 9 aa, Artificial Sequence
  peptide
YIGCLYTFV

SEQ ID NO: 161 - protein, 9 aa, Artificial Sequence
  peptide
YIVKPLPPV

SEQ ID NO: 162 - protein, 9 aa, Artificial Sequence
  peptide
YLCSWKPGV

SEQ ID NO: 163 - protein, 9 aa, Artificial Sequence
  peptide
YLDDGIWSI

SEQ ID NO: 164 - protein, 9 aa, Artificial Sequence
  peptide
YLDDGIWSL

SEQ ID NO: 165 - protein, 9 aa, Artificial Sequence
  peptide
YLDDGIWSV

SEQ ID NO: 166 - protein, 9 aa, Artificial Sequence
  peptide
YLDHALQCV

SEQ ID NO: 167 - protein, 9 aa, Artificial Sequence
  peptide
YLDKQCWEV

SEQ ID NO: 168 - protein, 9 aa, Artificial Sequence
  peptide
YLFYWYEGI

SEQ ID NO: 169 - protein, 9 aa, Artificial Sequence
  peptide
YLFYWYEGL

SEQ ID NO: 170 - protein, 9 aa, Artificial Sequence
  peptide
YLFYWYEGV

SEQ ID NO: 171 - protein, 9 aa, Artificial Sequence
  peptide
YLGCLYTFI

SEQ ID NO: 172 - protein, 9 aa, Artificial Sequence
  peptide
YLGCLYTFL

SEQ ID NO: 173 - protein, 9 aa, Artificial Sequence
  peptide
YLGCLYTFV

SEQ ID NO: 174 - protein, 9 aa, Artificial Sequence
  peptide
YLISTTFGI

SEQ ID NO: 175 - protein, 9 aa, Artificial Sequence
  peptide
YLISTTFGL

SEQ ID NO: 176 - protein, 9 aa, Artificial Sequence
  peptide
YLISTTFGV

SEQ ID NO: 177 - protein, 9 aa, Artificial Sequence
  peptide
YLNETYTLK

SEQ ID NO: 178 - protein, 9 aa, Artificial Sequence
  peptide
YLPFGFILV

SEQ ID NO: 179 - protein, 9 aa, Artificial Sequence
  peptide
YLQDMCVYY

SEQ ID NO: 180 - protein, 9 aa, Artificial Sequence
  peptide
YLSDYKDFY

SEQ ID NO: 181 - protein, 9 aa, Artificial Sequence
  peptide
YLTNYNLFY

SEQ ID NO: 182 - protein, 9 aa, Artificial Sequence
  peptide
YLVKPLPPI

SEQ ID NO: 183 - protein, 9 aa, Artificial Sequence
  peptide
YLVKPLPPL

SEQ ID NO: 184 - protein, 9 aa, Artificial Sequence
  peptide
YLVKPLPPV

SEQ ID NO: 185 - protein, 9 aa, Artificial Sequence
  peptide
YLWKTIITK

SEQ ID NO: 186 - protein, 9 aa, Artificial Sequence
  peptide
YLWQPPLSI

SEQ ID NO: 187 - protein, 9 aa, Artificial Sequence
  peptide
YLWQPPLSL

SEQ ID NO: 188 - protein, 9 aa, Artificial Sequence
  peptide
YLWQPPLSV

SEQ ID NO: 189 - protein, 9 aa, Artificial Sequence
  peptide
YLYLLCSWK

SEQ ID NO: 190 - protein, 9 aa, Artificial Sequence
  peptide
YLYTFLISI

SEQ ID NO: 191 - protein, 9 aa, Artificial Sequence
  peptide
YLYTFLISL

SEQ ID NO: 192 - protein, 9 aa, Artificial Sequence
  peptide
YLYTFLIST

SEQ ID NO: 193 - protein, 9 aa, Artificial Sequence
  peptide
YLYTFLISV

SEQ ID NO: 194 - protein, 9 aa, Artificial Sequence
  peptide
YMCSWKPGI

SEQ ID NO: 195 - protein, 9 aa, Artificial Sequence
  peptide
YMCSWKPGV

SEQ ID NO: 196 - protein, 9 aa, Artificial Sequence
  peptide
YMDDGIWSI

SEQ ID NO: 197 - protein, 9 aa, Artificial Sequence
  peptide
YMDDGIWSL

SEQ ID NO: 198 - protein, 9 aa, Artificial Sequence
  peptide
YMDDGIWSV

SEQ ID NO: 199 - protein, 9 aa, Artificial Sequence
  peptide
YMDHALQCV

SEQ ID NO: 200 - protein, 9 aa, Artificial Sequence
  peptide
YMDKQCWEV

SEQ ID NO: 201 - protein, 9 aa, Artificial Sequence
  peptide
YMFYWYEGI

SEQ ID NO: 202 - protein, 9 aa, Artificial Sequence
  peptide
YMFYWYEGL

SEQ ID NO: 203 - protein, 9 aa, Artificial Sequence
  peptide
YMFYWYEGV

SEQ ID NO: 204 - protein, 9 aa, Artificial Sequence
  peptide
YMGCLYTFI

SEQ ID NO: 205 - protein, 9 aa, Artificial Sequence
  peptide
YMGCLYTFL

SEQ ID NO: 206 - protein, 9 aa, Artificial Sequence
  peptide
YMGCLYTFV

SEQ ID NO: 207 - protein, 9 aa, Artificial Sequence
  peptide
YMISTTFGI

SEQ ID NO: 208 - protein, 9 aa, Artificial Sequence
  peptide
YMISTTFGL

SEQ ID NO: 209 - protein, 9 aa, Artificial Sequence
  peptide
YMISTTFGV

SEQ ID NO: 210 - protein, 9 aa, Artificial Sequence
  peptide
YMLAIGCLY

SEQ ID NO: 211 - protein, 9 aa, Artificial Sequence
  peptide
YMNETYTLK

SEQ ID NO: 212 - protein, 9 aa, Artificial Sequence
  peptide
YMPFGFILV

SEQ ID NO: 213 - protein, 9 aa, Artificial Sequence
  peptide
YMQDMCVYY

SEQ ID NO: 214 - protein, 9 aa, Artificial Sequence
  peptide
YMSDYKDFY

SEQ ID NO: 215 - protein, 9 aa, Artificial Sequence
  peptide
YMTGLLLRK

SEQ ID NO: 216 - protein, 9 aa, Artificial Sequence
  peptide
YMTNYNLFY

SEQ ID NO: 217 - protein, 9 aa, Artificial Sequence
  peptide
YMVIFVTGV

SEQ ID NO: 218 - protein, 9 aa, Artificial Sequence
  peptide
YMVKPLPPI

SEQ ID NO: 219 - protein, 9 aa, Artificial Sequence
  peptide
YMVKPLPPL

SEQ ID NO: 220 - protein, 9 aa, Artificial Sequence
  peptide
YMVKPLPPV

SEQ ID NO: 221 - protein, 9 aa, Artificial Sequence
  peptide
YMWKTIITK

SEQ ID NO: 222 - protein, 9 aa, Artificial Sequence
  peptide
YMWQPPLSI

SEQ ID NO: 223 - protein, 9 aa, Artificial Sequence
  peptide
YMWQPPLSL

SEQ ID NO: 224 - protein, 9 aa, Artificial Sequence
  peptide
YMWQPPLSV

SEQ ID NO: 225 - protein, 9 aa, Artificial Sequence
  peptide
YMYLLCSWK

SEQ ID NO: 226 - protein, 9 aa, Artificial Sequence
  peptide
YMYTFLISI

SEQ ID NO: 227 - protein, 9 aa, Artificial Sequence
  peptide
YMYTFLISL

SEQ ID NO: 228 - protein, 9 aa, Artificial Sequence
  peptide
YMYTFLIST

SEQ ID NO: 229 - protein, 9 aa, Artificial Sequence
  peptide
YMYTFLISV

SEQ ID NO: 230 - protein, 9 aa, Artificial Sequence
  peptide
YQWQPPLSV

SEQ ID NO: 231 - protein, 9 aa, Artificial Sequence
  peptide
YSDDGIWSI

SEQ ID NO: 232 - protein, 9 aa, Artificial Sequence
  peptide
YSDDGIWSL

SEQ ID NO: 233 - protein, 9 aa, Artificial Sequence
  peptide
YSDDGIWSV

SEQ ID NO: 234 - protein, 9 aa, Artificial Sequence
  peptide
YSDKQCWEI

SEQ ID NO: 235 - protein, 9 aa, Artificial Sequence
  peptide
YSDKQCWEL

SEQ ID NO: 236 - protein, 9 aa, Artificial Sequence
  peptide
YSDKQCWEV

SEQ ID NO: 237 - protein, 9 aa, Artificial Sequence
  peptide
YSDYKDFYI

SEQ ID NO: 238 - protein, 9 aa, Artificial Sequence
  peptide
YSDYKDFYL

SEQ ID NO: 239 - protein, 9 aa, Artificial Sequence
  peptide
YSDYKDFYV

SEQ ID NO: 240 - protein, 9 aa, Artificial Sequence
  peptide
YSSWAETTY

SEQ ID NO: 241 - protein, 9 aa, Artificial Sequence
  peptide
YTWKTIITK

SEQ ID NO: 242 - protein, 9 aa, Artificial Sequence
  peptide
YVQDMCVYY

SEQ ID NO: 243 - protein, 9 aa, Artificial Sequence
  peptide
AIGCLYTFL

SEQ ID NO: 244 - protein, 9 aa, Artificial Sequence
  peptide
ASDYKDFYI

SEQ ID NO: 245 - protein, 9 aa, Artificial Sequence
  peptide
CLYTFLIST

SEQ ID NO: 246 - protein, 9 aa, Artificial Sequence
  peptide
CSDDGIWSE

SEQ ID NO: 247 - protein, 9 aa, Artificial Sequence
  peptide
EASDYKDFY

SEQ ID NO: 248 - protein, 9 aa, Artificial Sequence
  peptide
ETWKTIITK

SEQ ID NO: 249 - protein, 9 aa, Artificial Sequence
  peptide
FLISTTFGC

SEQ ID NO: 250 - protein, 9 aa, Artificial Sequence
  peptide
FVTGLLLRK

SEQ ID NO: 251 - protein, 9 aa, Artificial Sequence
  peptide
GLDHALQCV

SEQ ID NO: 252 - protein, 9 aa, Artificial Sequence
  peptide
ILVIFVTGL

SEQ ID NO: 253 - protein, 9 aa, Artificial Sequence
  peptide
KVQDMCVYY

SEQ ID NO: 254 - protein, 9 aa, Artificial Sequence
  peptide
LDTNYNLFY

SEQ ID NO: 255 - protein, 9 aa, Artificial Sequence
  peptide
LLCSWKPGI

SEQ ID NO: 256 - protein, 9 aa, Artificial Sequence
  peptide
LQWQPPLSL

SEQ ID NO: 257 - protein, 9 aa, Artificial Sequence
  peptide
NIVKPLPPV

SEQ ID NO: 258 - protein, 9 aa, Artificial Sequence
  peptide
NLFYWYEGL

SEQ ID NO: 259 - protein, 9 aa, Artificial Sequence
  peptide
QSSWAETTY

SEQ ID NO: 260 - protein, 9 aa, Artificial Sequence
  peptide
RNIGSETWK

SEQ ID NO: 261 - protein, 9 aa, Artificial Sequence
  peptide
VCLAIGCLY

SEQ ID NO: 262 - protein, 9 aa, Artificial Sequence
  peptide
VENETYTLK

SEQ ID NO: 263 - protein, 9 aa, Artificial Sequence
  peptide
WLPFGFILI

SEQ ID NO: 264 - protein, 9 aa, Artificial Sequence
  peptide
WQYLLCSWK

SEQ ID NO: 265 - protein, 9 aa, Artificial Sequence
  peptide
WSDKQCWEG

SEQ ID NO: 266 - protein, 20 aa, Artificial Sequence
  peptide
MAKTIAYDEEARRGLERGLN

SEQ ID NO: 267 - protein, 9 aa, Artificial Sequence
  peptide
YLPFGFILV

SEQ ID NO: 268 - protein, 9 aa, Artificial Sequence
  peptide
VLPFGFILV

SEQ ID NO: 269 - protein, 9 aa, Artificial Sequence
  peptide
NLPFGFILV

SEQ ID NO: 270 - protein, 9 aa, Artificial Sequence
  peptide
RLPFGFILV

SEQ ID NO: 271 - protein, 9 aa, Artificial Sequence
  peptide
SLPFGFILV

SEQ ID NO: 272 - protein, 9 aa, Artificial Sequence
  peptide
TLPFGFILV

SEQ ID NO: 273 - protein, 9 aa, Artificial Sequence
  peptide
CLPFGFILV

SEQ ID NO: 274 - protein, 9 aa, Artificial Sequence
  peptide
LLPFGFILV

SEQ ID NO: 275 - protein, 380 aa, Homo sapiens
MAFVCLAIGCLYTFLISTTFGCTSSSDTEIKVNPPQDFEIVDPGYLGYLYLQWQPPLSLDHFKECTVEYELKYRNIGSETWKTIITKNLHYKDGFDLNKGIEAKIHTLLPWQCTNGSEVQSSWAETTYWISPQGIPETKVQDMDCVYYNWQYLLCSWKPGIGVLLDTNYNLFYWYEGLDHALQCVDYIKADGQNIGCRFPYLEASDYKDFYICVNGSSENKPIRSSYFTFQLQNIVKPLPPVYLTFTRESSCEIKLKWSIPLGPIPARCFDYEIEIREDDTTLVTATVENETYTLKTTNETRQLCFVVRSKVNIYCSDDGIWSEWSDKQCWEGEDLSKKTLLRFWLPFGFILILVIFVTGLLLRKPNTYPKMIPEFFCDT

SEQ ID NO: 276 - protein, 10 aa, Artificial Sequence
  peptide
WLPFGFILIL

SEQ ID NO: 277 - protein, 9 aa, Artificial Sequence
  peptide
VLLDTNYNL

SEQ ID NO: 278 - protein, 9 aa, Artificial Sequence
  peptide
GLDHALQCV

SEQ ID NO: 279 - protein, 10 aa, Artificial Sequence
  peptide
FLPFGFILPV

SEQ ID NO: 280 - protein, 13 aa, Artificial Sequence
  peptide
TPPAYRPPNAPIL

SEQ ID NO: 281 - protein, 15 aa, Artificial Sequence
  peptide
KSVWSKLQSIGIRQH

SEQ ID NO: 282 - protein, 9 aa, Artificial Sequence
  peptide
ALPFGFILV

SEQ ID NO: 283 - protein, 9 aa, Artificial Sequence
  peptide
WLPFGFILV

SEQ ID NO: 284 - protein, 9 aa, Artificial Sequence
  peptide
ELPFGFILV

SEQ ID NO: 285 - protein, 142 aa, Homo sapiens
MGAPTLPPAWQPFLKDHRISTFKNWPFLEGCACTPERMAEAGFIHCPTENEPDLAQCFFCFKELEGWEPDDDPIEEHKKHSSGCAFLSVKKQFEELTLGEFLKLDRERAKNKIAKETNNKKKEFEETAKKVRRAIEQLAAMD

SEQ ID NO: 286 - protein, 9 aa, Homo sapiens
LTLGEFLKL

SEQ ID NO: 287 - protein, 9 aa, Artificial Sequence
  peptide
YTLGEFLYI

SEQ ID NO: 288 - protein, 9 aa, Artificial Sequence
  peptide
GLLGEFLQI

SEQ ID NO: 289 - protein, 9 aa, Artificial Sequence
  peptide
FMLGEFLKL

SEQ ID NO: 290 - protein, 763 aa, Homo sapiens
MKTSPRRPLILKRRRLPLPVQNAPSETSEEEPKRSPAQQESNQAEASKEVAESNSCKFPAGIKIINHPTMPNTQVVAIPNNANIHSIITALTAKGKESGSSGPNKFILISCGGAPTQPPGLRPQTQTSYDAKRTEVTLETLGPKPAARDVNLPRPPGALCEQKRETCADGEAAGCTINNSLSNIQWLRKMSSDGLGSRSIKQEMEEKENCHLEQRQVKVEEPSRPSASWQNSVSERPPYSYMAMIQFAINSTERKRMTLKDIYTWIEDHFPYFKHIAKPGWKNSIRHNLSLHDMFVRETSANGKVSFWTIHPSANRYLTLDQVFKPLDPGSPQLPEHLESQQKRPNPELRRNMTIKTELPLGARRKMKPLLPRVSSYLVPIQFPVNQSLVLQPSVKVPLPLAASLMSSELARHSKRVRIAPKVLLAEEGIAPLSSAGPGKEEKLLFGEGFSPLLPVQTIKEEEIQPGEEMPHLARPIKVESPPLEEWPSPAPSFKEESSHSWEDSSQSPTPRPKKSYSGLRSPTRCVSEMLVIQHRERRERSRSRRKQHLLPPCVDEPELLFSEGPSTSRWAAELPFPADSSDPASQLSYSQEVGGPFKTPIKETLPISSTPSKSVLPRTPESWRLTPPAKVGGLDFSPVQTSQGASDPLPDPLGLMDLSTTPLQSAPPLESPQRLLSSEPLDLISVPFGNSSPSDIDVPKPGSPEPQVSGLAANRSLTEGLVLDTMNDSLSKILLDISFPGLDEDPLGPDNINWSQFIPELQ

SEQ ID NO: 291 - protein, 9 aa, Homo sapiens
ILLDISFPG

SEQ ID NO: 292 - protein, 9 aa, Homo sapiens
LLDISFPGL

SEQ ID NO: 293 - protein, 9 aa, Homo sapiens
LMDLSTTPL

SEQ ID NO: 294 - protein, 9 aa, Homo sapiens
RVSSYLVPI

SEQ ID NO: 295 - protein, 9 aa, Homo sapiens
SLSKILLDI

SEQ ID NO: 296 - protein, 9 aa, Homo sapiens
SQLSYSQEV

SEQ ID NO: 297 - protein, 9 aa, Homo sapiens
WAAELPFPA

SEQ ID NO: 298 - protein, 9 aa, Homo sapiens
NLSLHDMFV

SEQ ID NO: 299 - protein, 9 aa, Homo sapiens
KMKPLLPRV

SEQ ID NO: 300 - protein, 9 aa, Homo sapiens
YLVPIQFPV

SEQ ID NO: 301 - protein, 9 aa, Homo sapiens
YMAMIQFAI

SEQ ID NO: 302 - protein, 9 aa, Artificial Sequence
  peptide
TLLDISFAA

SEQ ID NO: 303 - protein, 9 aa, Artificial Sequence
  peptide
NMLDISFYL

SEQ ID NO: 304 - protein, 9 aa, Artificial Sequence
  peptide
WLLDISFPL

SEQ ID NO: 305 - protein, 9 aa, Artificial Sequence
  peptide
HLLDISFPA

SEQ ID NO: 306 - protein, 9 aa, Artificial Sequence
  peptide
ELLDISFPA

SEQ ID NO: 307 - protein, 9 aa, Artificial Sequence
  peptide
VLLDISFEL

SEQ ID NO: 308 - protein, 9 aa, Artificial Sequence
  peptide
VLLDISFKV

SEQ ID NO: 309 - protein, 9 aa, Artificial Sequence
  peptide
IMLDISFLL

SEQ ID NO: 310 - protein, 9 aa, Artificial Sequence
  peptide
ILDISFPLV

SEQ ID NO: 311 - protein, 9 aa, Artificial Sequence
  peptide
LLDISFPSL

SEQ ID NO: 312 - protein, 9 aa, Artificial Sequence
  peptide
LMDLSTTEV

SEQ ID NO: 313 - protein, 9 aa, Artificial Sequence
  peptide
LMDLSTTNV

SEQ ID NO: 314 - protein, 9 aa, Artificial Sequence
  peptide
RLSSYLVEI

SEQ ID NO: 315 - protein, 9 aa, Artificial Sequence
  peptide
MVSSYLVEV

SEQ ID NO: 316 - protein, 9 aa, Artificial Sequence
  peptide
KVSSYLVEV

SEQ ID NO: 317 - protein, 9 aa, Artificial Sequence
  peptide
MLSSYLVPI

SEQ ID NO: 318 - protein, 9 aa, Artificial Sequence
  peptide
LLSSYLVPI

SEQ ID NO: 319 - protein, 9 aa, Artificial Sequence
  peptide
FVSSYLVPT

SEQ ID NO: 320 - protein, 9 aa, Artificial Sequence
  peptide
ILSKILLFA

SEQ ID NO: 321 - protein, 9 aa, Artificial Sequence
  peptide
YQLSYSQMV

SEQ ID NO: 322 - protein, 9 aa, Artificial Sequence
  peptide
KLLSYSQEL

SEQ ID NO: 323 - protein, 9 aa, Artificial Sequence
  peptide
KIAELPFPL

SEQ ID NO: 324 - protein, 9 aa, Artificial Sequence
  peptide
SLSLHDMFL

SEQ ID NO: 325 - protein, 9 aa, Artificial Sequence
  peptide
KLKPLLPWI

SEQ ID NO: 326 - protein, 9 aa, Artificial Sequence
  peptide
KLKPLLPFL

SEQ ID NO: 327 - protein, 9 aa, Artificial Sequence
  peptide
KVVPIQFPV

SEQ ID NO: 328 - protein, 9 aa, Artificial Sequence
  peptide
KIVPIQFPI

SEQ ID NO: 329 - protein, 9 aa, Artificial Sequence
  peptide
YQAMIQFLI

SEQ ID NO: 330 - protein, 9 aa, Artificial Sequence
  peptide
LMLGEFLKL

SEQ ID NO: 331 - protein, 10 aa, Homo sapiens
FLISTTFGCT

SEQ ID NO: 332 - protein, 10 aa, Homo sapiens
YLYLQWQPPL

SEQ ID NO: 333 - protein, 10 aa, Homo sapiens
GVLLDTNYNL

SEQ ID NO: 334 - protein, 10 aa, Homo sapiens
FQLQNIVKPL

SEQ ID NO: 335 - protein, 10 aa, Artificial Sequence
  peptide
FMPFGFILPI

SEQ ID NO: 336 - protein, 10 aa, Artificial Sequence
  peptide
FMPFGFILGV

SEQ ID NO: 337 - protein, 10 aa, Artificial Sequence
  peptide
FLISTTFTIN

SEQ ID NO: 338 - protein, 10 aa, Artificial Sequence
  peptide
FMISTTFMRL

SEQ ID NO: 339 - protein, 10 aa, Artificial Sequence
  QMISTTFGNV
QMISTTFGNV

SEQ ID NO: 340 - protein, 10 aa, Artificial Sequence
  peptide
WLYLQWQPSV

SEQ ID NO: 341 - protein, 10 aa, Artificial Sequence
  peptide
FVLLDTNYEI

SEQ ID NO: 342 - protein, 10 aa, Artificial Sequence
  peptide
FILLDTNYEI

SEQ ID NO: 343 - protein, 10 aa, Artificial Sequence
  peptide
YELQNIVLPI

SEQ ID NO: 344 - protein, 10 aa, Artificial Sequence
  peptide
FMLQNIVKNL